European Patent Application EP 4 653 001 A1, published November 26, 2025. Title: TREATMENT, DIAGNOSIS AND/OR PROGNOSIS OF MITOCHONDRIAL DISEASES. Applicant: UNIVERSIDAD AUTÓNOMA DE MADRID. The sequence listing filed with the application follows.

SEQUENCE LISTING (7 sequences)

SEQ ID NO: 1 - DNA, 20 bp, synthetic construct
  source 1..20: mol_type = other DNA
ttggaatagctcatacccgt

SEQ ID NO: 2 - DNA, 20 bp, synthetic construct
  source 1..20: mol_type = other DNA
cttgaaggtgaggataacgc

SEQ ID NO: 3 - DNA, 20 bp, synthetic construct
  source 1..20: mol_type = other DNA
gacacacctacctgtcgtgg

SEQ ID NO: 4 - DNA, 20 bp, synthetic construct
  source 1..20: mol_type = other DNA
tgtcaaagaatagcaacaga

SEQ ID NO: 5 - DNA, 19 bp, synthetic construct
  source 1..19: mol_type = other DNA
caggcccggaacacacgga

SEQ ID NO: 6 - DNA, 20 bp, synthetic construct
  source 1..20: mol_type = other DNA
gccagcgggagcacatcggt

SEQ ID NO: 7 - DNA, 20 bp, synthetic construct
  source 1..20: mol_type = other DNA
atagagccaatttacccaca